European Patent Specification EP 3 556 766 B1, published July 31, 2024. Title: Cell membrane penetrating peptide and intracellular delivery carrier comprising thereof. Applicant: Avixgen Incorporation. The sequence listing filed with the application follows.

SEQUENCE LISTING (23 sequences)

SEQ ID NO: 1 - DNA, 19 bp, Artificial Sequence
  synthetic polynucleotide
catatgcagcggggaactt

SEQ ID NO: 2 - DNA, 19 bp, Artificial Sequence
  synthetic polynucleotide
tccggagtttgcctgtctc

SEQ ID NO: 3 - DNA, 20 bp, Artificial Sequence
  synthetic polynucleotide
tccggagtgagcaagggcga

SEQ ID NO: 4 - DNA, 21 bp, Artificial Sequence
  synthetic polynucleotide
aagcttcttgtacactctcgt

SEQ ID NO: 5 - protein, 6 aa, Artificial Sequence
  hexapeptide
EEMQRR

SEQ ID NO: 6 - protein, 11 aa, Artificial Sequence
  PTD-ys peptide
YARVRRRGPRR

SEQ ID NO: 7 - protein, 12 aa, Artificial Sequence
  TLM peptide
PLSSIFSRIGDP

SEQ ID NO: 8 - protein, 13 aa, Artificial Sequence
  TD1 peptide
KAMININKFLNQC

SEQ ID NO: 9 - protein, 45 aa, Artificial Sequence
  NC-hexapeptide
VKCFNCGKEGHTARNCRAPRKKGCWKCGKEGHQMKDCTEEEMQRR

SEQ ID NO: 10 - protein, 23 aa, Artificial Sequence
  13NC35 peptide
VKCFNCGKEGHTARNCRAPRKKG

SEQ ID NO: 11 - protein, 22 aa, Artificial Sequence
  29NC50 peptide
RAPRKKGCWKCGKEGHQMKDCT

SEQ ID NO: 12 - protein, 55 aa, Artificial Sequence
  HIV-NC peptide
MQRGNFRNQRKIVKCFNCGKEGHTARNCRAPRKKGCWKCGKEGHQMKDCTERQAN

SEQ ID NO: 13 - protein, 42 aa, Artificial Sequence
  SIV-NC peptide
RGPLKCFNCGKFGHMQRECKAPRQIKCFKCGKIGHMAKDCKN

SEQ ID NO: 14 - protein, 63 aa, Artificial Sequence
  RSV-NC peptide
GQTGSGGRARGLCYTCGSPGHYQAQCPKKRKSGNSRERCQLCDGMGHNAKQCRKRDGNQGQRP

SEQ ID NO: 15 - protein, 56 aa, Artificial Sequence
  MLV-NC peptide
ATVVSGQKQDRQGGERRRSQLDRDQCAYCKEKGHWAKDCPKKPRGPRGPRPQTSLL

SEQ ID NO: 16 - protein, 14 aa, Artificial Sequence
  synthetic polypeptide
  UNSURE (2): Ala, Val, Ile, Leu, Met, Phe, Tyr, Trp, Ser, Thr, Asn or Gln
  UNSURE (3): Ala, Val, Ile, Leu, Met, Phe, Tyr, Trp, Arg, His, Lys, Asn, Ser, Thr or Gln
  UNSURE (5): Asp, Glu, Arg, His, Lys, Ser, Thr, Asn, Gln or Gly
  UNSURE (6): Asp, Glu, Arg, His, Lys, Ser, Thr, Asn, Gln or Gly
  UNSURE (7): Asp, Glu, Arg, His, Lys, Ala, Val, Ile, Leu, Met, Phe, Tyr, Trp or Pro
  UNSURE (10): Ser, Thr, Asn, Gln, Ala, Val, Ile, Leu, Met, Phe, Tyr or Trp
  UNSURE (11): Ser, Thr, Asn, Gln, Ala, Val, Ile, Leu, Met, Phe, Tyr or Trp
  UNSURE (12): Lys, Ala or Arg
  UNSURE (13): Asp, Glu, Ser, Thr, Asn or Gln
CXXCXXXGHXXXXC

SEQ ID NO: 17 - protein, 14 aa, Artificial Sequence
  HIV-NC 1st zinc finger domain
CFNCGKEGHTARNC

SEQ ID NO: 18 - protein, 14 aa, Artificial Sequence
  HIV-NC 2nd zinc finger domain
CWKCGKEGHQMKDC

SEQ ID NO: 19 - protein, 14 aa, Artificial Sequence
  SIV-NC 1st zinc finger domain
CFNCGKEGHMQREC

SEQ ID NO: 20 - protein, 14 aa, Artificial Sequence
  SIV-NC 2nd zinc finger domain
CFKCGKIGHMAKDC

SEQ ID NO: 21 - protein, 14 aa, Artificial Sequence
  RSV-NC 1st zinc finger domain
CYTCGSPGHYQAQC

SEQ ID NO: 22 - protein, 14 aa, Artificial Sequence
  RSV-NC 2nd zinc finger domain
CQLCDGMGHNAKQC

SEQ ID NO: 23 - protein, 14 aa, Artificial Sequence
  MLV-NC zinc finger domain
CAYCKEKGHWAKDC